European Patent Application EP 4 606 894 A1, published August 27, 2025. Title: Cas 단백질 및 박테리아 톡신을 포함하는 융합 단백질 및 이의 용도. Applicant: 성균관대학교산학협력단. The sequence listing filed with the application follows.

SEQUENCE LISTING (45 sequences)

SEQ ID NO: 1 - protein, 410 aa, synthetic construct
MSAAARVNDPIEHTGSLTGLLAGLAIGAIGAALVVGTGGLAAVAIVGASAATGAGVGQLIGSLSCCNHQTGQIVSGSSNVYINGEPAARAHADQAKCDEHTSRPQVIAQGSSNVYINGHPAARVGDRTACDAKIVVGSSNVFIGGGTETTDPINPEVPELLERSILLVGLASAVVLASPVIVIAGLVGGIAGGTVGSMGGAQLFGEGTDGQKLMAFGGALLGGGLGAKGGKWFDTRYDIKVQGVGSNLGNLKITPKGAAKVSNIAESEAALGRASQARADLPQSKELKVKTVSSNDKKTLSGWGNKKPEGYERISAEQVKAKSEEIGHEVKSHPYDRDYKGQYFSSHAEKQMSIASPNHPLGVSKPMCTDCQGYFSQLAKYSKVEQTVADPKAIRIFKTDGSVETIMRSE

SEQ ID NO: 2 - protein, 151 aa, synthetic construct
KVSNIAESEAALGRASQARADLPQSKELKVKTVSSNDKKTLSGWGNKKPEGYERISAEQVKAKSEEIGHEVKSHPYDRDYKGQYFSSHAEKQMSIASPNHPLGVSKPMCTDCQGYFSQLAKYSKVEQTVADPKAIRIFKTDGSVETIMRSE

SEQ ID NO: 3 - protein, 193 aa, synthetic construct
MNNKSKVLIEKLLLEVAKSPEGELILPLRKLLWNTITEDETAAKKKAILTALDVMCVRQGVNFWIKKFGDNEPLNYILNIALETAEGKFDESKALGLRDEFYVSIVEDQEYEVEEYPAMFVGHAAANTIARAVDDFQFEPYDHRVDRDLDPEGFESSYLVASAFAGGLSEDGDPKLRRAFWEWYLSIAVPQVV

SEQ ID NO: 4 - DNA, 35 bp, synthetic construct
  source 1..35: mol_type = other DNA
aaaaaaaaaaaaaaagcgaaaaaaaaaaaaaaaaa

SEQ ID NO: 5 - DNA, 23 bp, synthetic construct
  source 1..23: mol_type = other DNA
gtcatcttagtcattacctgagg

SEQ ID NO: 6 - DNA, 23 bp, synthetic construct
  source 1..23: mol_type = other DNA
gaacacaaagcatagactgcggg

SEQ ID NO: 7 - RNA, 21 nt, synthetic construct
  source 1..21: mol_type = other RNA
gtctacagacatagaggattt

SEQ ID NO: 8 - DNA, 39 bp, synthetic construct
  source 1..39: mol_type = other DNA
ggaaactggaacacaaagcatagactgcggggcgggcca

SEQ ID NO: 9 - DNA, 39 bp, synthetic construct
  source 1..39: mol_type = other DNA
ggaaactggaacataaagcatagactgcggggcgggcca

SEQ ID NO: 10 - DNA, 39 bp, synthetic construct
  source 1..39: mol_type = other DNA
ggaaactggaatataaagcatagactgcggggcgggcca

SEQ ID NO: 11 - DNA, 39 bp, synthetic construct
  source 1..39: mol_type = other DNA
ggaaactggaatacaaagcatagactgcggggcgggcca

SEQ ID NO: 12 - DNA, 39 bp, synthetic construct
  source 1..39: mol_type = other DNA
ggaaactggaacacaaagtatagactgcggggcgggcca

SEQ ID NO: 13 - DNA, 75 bp, synthetic construct
  source 1..75: mol_type = other DNA
aattttccagcccgctggccctgtaaaggaaactggaacacaaagcatagactgcggggcgggccagcctgaata

SEQ ID NO: 14 - DNA, 18 bp, synthetic construct
  source 1..18: mol_type = other DNA
aattttccagcctgaata

SEQ ID NO: 15 - DNA, 66 bp, synthetic construct
  source 1..66: mol_type = other DNA
aattttccagcccgctggccctgtaaaggaaactggaacacaaagcggggcgggccagcctgaata

SEQ ID NO: 16 - DNA, 49 bp, synthetic construct
  source 1..49: mol_type = other DNA
aattttccagcccgctggccctgtaaaggaaactggaacacaaagcata

SEQ ID NO: 17 - protein, 151 aa, synthetic construct
KVSNIAESEAALGRASQARADLPQSKELKVKTVSSNDKKTLSDWGNKKPEGYERISAEQVKAKSEEIGHEVKSHPYDRDYKGQYFSSHAEKQMSIASPNHPLGVSKPMCTDCQGYFSQLAKYSKVEQTVADPKAIRIFKTDGSVETIMRSE

SEQ ID NO: 18 - DNA, 20 bp, synthetic construct
  source 1..20: mol_type = other DNA
gaacacaaagcatagactgc

SEQ ID NO: 19 - DNA, 20 bp, synthetic construct
  source 1..20: mol_type = other DNA
ccagcccgctggccctgtaa

SEQ ID NO: 20 - DNA, 20 bp, synthetic construct
  source 1..20: mol_type = other DNA
gctggccctgtaaaggaaac

SEQ ID NO: 21 - DNA, 20 bp, synthetic construct
  source 1..20: mol_type = other DNA
gtttcctttacagggccagc

SEQ ID NO: 22 - DNA, 20 bp, synthetic construct
  source 1..20: mol_type = other DNA
gcacttgtttgcagctattc

SEQ ID NO: 23 - DNA, 20 bp, synthetic construct
  source 1..20: mol_type = other DNA
ggcccagactgagcacgtga

SEQ ID NO: 24 - DNA, 20 bp, synthetic construct
  source 1..20: mol_type = other DNA
ctgcttctccagccctggcc

SEQ ID NO: 25 - DNA, 20 bp, synthetic construct
  source 1..20: mol_type = other DNA
ccctggcctgggtcaatcct

SEQ ID NO: 26 - DNA, 20 bp, synthetic construct
  source 1..20: mol_type = other DNA
gactgagcacgtgatggcag

SEQ ID NO: 27 - DNA, 20 bp, synthetic construct
  source 1..20: mol_type = other DNA
cttcctccagagggcgtcgc

SEQ ID NO: 28 - DNA, 20 bp, synthetic construct
  source 1..20: mol_type = other DNA
caggacagcttttcctagac

SEQ ID NO: 29 - DNA, 20 bp, synthetic construct
  source 1..20: mol_type = other DNA
cagctcctgcaccgggatac

SEQ ID NO: 30 - DNA, 20 bp, synthetic construct
  source 1..20: mol_type = other DNA
ggcactgcggctggaggtgg

SEQ ID NO: 31 - DNA, 20 bp, synthetic construct
  source 1..20: mol_type = other DNA
ggggcaccgcggcgccccgg

SEQ ID NO: 32 - DNA, 20 bp, synthetic construct
  source 1..20: mol_type = other DNA
gcggcgccccggtggcactg

SEQ ID NO: 33 - DNA, 20 bp, synthetic construct
  source 1..20: mol_type = other DNA
cgccccggtggcactgcggc

SEQ ID NO: 34 - DNA, 20 bp, synthetic construct
  source 1..20: mol_type = other DNA
tcccttccttccacccagcc

SEQ ID NO: 35 - DNA, 20 bp, synthetic construct
  source 1..20: mol_type = other DNA
ccctgcctgtcatcctgctt

SEQ ID NO: 36 - DNA, 20 bp, synthetic construct
  source 1..20: mol_type = other DNA
gcagtgccaccggggcgccg

SEQ ID NO: 37 - DNA, 20 bp, synthetic construct
  source 1..20: mol_type = other DNA
ctccagccgcagtgccaccg

SEQ ID NO: 38 - DNA, 20 bp, synthetic construct
  source 1..20: mol_type = other DNA
acctccagccgcagtgccac

SEQ ID NO: 39 - DNA, 20 bp, synthetic construct
  source 1..20: mol_type = other DNA
gtcatcttagtcattacctg

SEQ ID NO: 40 - DNA, 20 bp, synthetic construct
  source 1..20: mol_type = other DNA
tacacgtctcatatgcccct

SEQ ID NO: 41 - DNA, 20 bp, synthetic construct
  source 1..20: mol_type = other DNA
tcaaccattaagcaaaacat

SEQ ID NO: 42 - DNA, 20 bp, synthetic construct
  source 1..20: mol_type = other DNA
gtcacctccaatgactaggg

SEQ ID NO: 43 - DNA, 20 bp, synthetic construct
  source 1..20: mol_type = other DNA
ggaatcccttctgcagcacc

SEQ ID NO: 44 - DNA, 20 bp, synthetic construct
  source 1..20: mol_type = other DNA
ggccacactagcgttgctgc

SEQ ID NO: 45 - DNA, 20 bp, synthetic construct
  source 1..20: mol_type = other DNA
tgacatcaattattatacat